European Patent Application EP 4 556 487 A1, published May 21, 2025. Title: GLP-1/GIP DUAL AGONIST, PREPARATION METHOD AND USE THEREOF. Applicant: 杭州中美华东制药有限公司. The sequence listing filed with the application follows.

SEQUENCE LISTING (13 sequences)

SEQ ID NO: 1 - protein, 40 aa, synthetic construct
  MOD_RES 2: note = Aib
  MOD_RES 6: note = alpha methyl phenylalanine
  MOD_RES 11: note = Aib
  MOD_RES 13: note = Aib
  MOD_RES 40: note = amidated
YXEGTXTSDYXIXLDKQAQAEFVKWLLKGGPSSGAPPPSK

SEQ ID NO: 2 - protein, 40 aa, synthetic construct; identical to SEQ ID NO: 1
  MOD_RES 2: note = Aib
  MOD_RES 6: note = alpha methyl phenylalanine
  MOD_RES 11: note = Aib
  MOD_RES 13: note = Aib
  MOD_RES 40: note = amidated
  SITE 24: note = the epsilon-amino of the K side-chain is conjugated with ([2-(2-amino-ethoxy)-ethoxy]-acetyl)2-(gama-Glu)1-CO-(CH2)16-CO2H

SEQ ID NO: 3 - protein, 40 aa, synthetic construct; identical to SEQ ID NO: 1
  MOD_RES 2: note = Aib
  MOD_RES 6: note = alpha methyl phenylalanine
  MOD_RES 11: note = Aib
  MOD_RES 13: note = Aib
  MOD_RES 40: note = amidated
  SITE 28: note = the epsilon-amino of the K side-chain is conjugated with ([2-(2-amino-ethoxy)-ethoxy]-acetyl)2-(gama-Glu)1-CO-(CH2)16-CO2H

SEQ ID NO: 4 - protein, 40 aa, synthetic construct; identical to SEQ ID NO: 1
  MOD_RES 2: note = Aib
  MOD_RES 6: note = alpha methyl phenylalanine
  MOD_RES 11: note = Aib
  MOD_RES 13: note = Aib
  MOD_RES 40: note = amidated
  SITE 24: note = the epsilon-amino of the K side-chain is conjugatged with ([2-(2-amino-ethoxy)-ethoxy]-acetyl)2-(gama-Glu)1-CO-(CH2)18-CO2H

SEQ ID NO: 5 - protein, 40 aa, synthetic construct; identical to SEQ ID NO: 1
  MOD_RES 2: note = Aib
  MOD_RES 6: note = alpha methyl phenylalanine
  MOD_RES 11: note = Aib
  MOD_RES 13: note = Aib
  MOD_RES 40: note = amidated
  SITE 24: note = the epsilon-amino of the K side-chain is conjugated with ([2-(2-amino-ethoxy)-ethoxy]-acetyl)2-(gama-Glu)1-CO-(CH2)20-CO2H

SEQ ID NO: 6 - protein, 40 aa, synthetic construct; identical to SEQ ID NO: 1
  MOD_RES 2: note = Aib
  MOD_RES 6: note = alpha methyl phenylalanine
  MOD_RES 11: note = Aib
  MOD_RES 13: note = Aib
  MOD_RES 40: note = amidated
  SITE 24: note = the epsilon-amino of the K side-chain is conjugated with ([2-(2-amino-ethoxy)-ethoxy]-acetyl)2-(gama-Glu)3-CO-(CH2)16-CO2H

SEQ ID NO: 7 - protein, 40 aa, synthetic construct; identical to SEQ ID NO: 1
  MOD_RES 2: note = Aib
  MOD_RES 6: note = alpha methyl phenylalanine
  MOD_RES 11: note = Aib
  MOD_RES 13: note = Aib
  MOD_RES 40: note = amidated
  SITE 24: note = the epsilon-amino of the K side-chain is conjugated with ([2-(2-amino-ethoxy)-ethoxy]-acetyl)3-(gama-Glu)1-CO-(CH2)20-CO2H

SEQ ID NO: 8 - protein, 40 aa, synthetic construct; identical to SEQ ID NO: 1
  MOD_RES 2: note = Aib
  MOD_RES 6: note = alpha methyl phenylalanine
  MOD_RES 11: note = Aib
  MOD_RES 13: note = Aib
  MOD_RES 40: note = amidated
  SITE 28: note = the epsilon-amino of the K side-chain is conjugated with ([2-(2-amino-ethoxy)-ethoxy]-acetyl)2-(gama-Glu)1-CO-(CH2)20-CO2H

SEQ ID NO: 9 - protein, 40 aa, synthetic construct; identical to SEQ ID NO: 1
  MOD_RES 2: note = Aib
  MOD_RES 6: note = alpha methyl phenylalanine
  MOD_RES 11: note = Aib
  MOD_RES 13: note = Aib
  MOD_RES 40: note = amidated
  SITE 28: note = the epsilon-amino of the K side-chain is conjugated with ([2-(2-amino-ethoxy)-ethoxy]-acetyl)2-(gama-Glu)3-CO-(CH2)16-CO2H

SEQ ID NO: 10 - protein, 40 aa, synthetic construct; identical to SEQ ID NO: 1
  MOD_RES 2: note = Aib
  MOD_RES 6: note = alpha methyl phenylalanine
  MOD_RES 11: note = Aib
  MOD_RES 13: note = Aib
  MOD_RES 40: note = amidated
  SITE 28: note = the epsilon-amino of the K side-chain is conjugated with ([2-(2-amino-ethoxy)-ethoxy]-acetyl)3-(gama-Glu)1-CO-(CH2)16-CO2H

SEQ ID NO: 11 - protein, 40 aa, synthetic construct; identical to SEQ ID NO: 1
  MOD_RES 2: note = Aib
  MOD_RES 6: note = alpha methyl phenylalanine
  MOD_RES 11: note = Aib
  MOD_RES 13: note = Aib
  MOD_RES 40: note = amidated
  SITE 28: note = the epsilon-amino of the K side-chain is conjugated with ([2-(2-amino-ethoxy)-ethoxy]-acetyl)3-(gama-Glu)1-CO-(CH2)20-CO2H

SEQ ID NO: 12 - protein, 40 aa, synthetic construct; identical to SEQ ID NO: 1
  MOD_RES 2: note = Aib
  MOD_RES 6: note = alpha methyl phenylalanine
  MOD_RES 11: note = Aib
  MOD_RES 13: note = Aib
  MOD_RES 40: note = amidated
  SITE 24: note = the epsilon-amino of the K side-chain may be conjugated with ([2-(2-amino-ethoxy)-ethoxy]-acetyl)a-(gama-Glu)b-CO-(CH2)c-Z, wherein each a is independently an integer from 0 to 5, each b is independently an integer from 0 to 5, and each c is independently an integer from 10 to 24, wherein Z is independently selected from the group consisting of -CH3, carboxylic acids or carboxylic acid bioisosteres, phosphonates or sulfonates
  SITE 16: note = the epsilon-amino of the K side-chain may be conjugated with ([2-(2-amino-ethoxy)-ethoxy]-acetyl)a-(gama-Glu)b-CO-(CH2)c-Z, wherein each a is independently an integer from 0 to 5, each b is independently an integer from 0 to 5, and each c is independently an integer from 10 to 24, wherein Z is independently selected from the group consisting of -CH3, carboxylic acids or carboxylic acid bioisosteres, phosphonates or sulfonates
  SITE 28: note = the epsilon-amino of the K side-chain may be conjugated with ([2-(2-amino-ethoxy)-ethoxy]-acetyl)a-(gama-Glu)b-CO-(CH2)c-Z, wherein each a is independently an integer from 0 to 5, each b is independently an integer from 0 to 5, and each c is independently an integer from 10 to 24, wherein Z is independently selected from the group consisting of -CH3, carboxylic acids or carboxylic acid bioisosteres, phosphonates or sulfonates
  SITE 40: note = the epsilon-amino of the K side-chain may be conjugated with ([2-(2-amino-ethoxy)-ethoxy]-acetyl)a-(gama-Glu)b-CO-(CH2)c-Z, wherein each a is independently an integer from 0 to 5, each b is independently an integer from 0 to 5, and each c is independently an integer from 10 to 24, wherein Z is independently selected from the group consisting of -CH3, carboxylic acids or carboxylic acid bioisosteres, phosphonates or sulfonates

SEQ ID NO: 13 - protein, 40 aa, synthetic construct
  MOD_RES 2: note = Aib
  MOD_RES 6: note = alpha methyl phenylalanine
  MOD_RES 11: note = Aib or Ala
  MOD_RES 13: note = Aib, cyclohexylalanine, Leu, alpha methyl phenylalanine or alpha methyl tyrosine
  SITE 24: note = the epsilon-amino of the K side-chain may be conjugated with ([2-(2-amino-ethoxy)-ethoxy]-acetyl)a-(gama-Glu)b-CO-(CH2)c-Z, wherein each a is independently an integer from 0 to 5, each b is independently an integer from 0 to 5, and each c is independently an integer from 10 to 24, wherein Z is independently selected from the group consisting of -CH3, carboxylic acids or carboxylic acid bioisosteres, phosphonates or sulfonates
  MOD_RES 12: note = Ala, Ile, Lys, Phe or 4-pyridinyl alanine
  MOD_RES 17: note = Gln or Ile
  MOD_RES 20: note = Ala or Ser
  MOD_RES 29: note = Gln or Gly
  SITE 16: note = the epsilon-amino of the K side-chain may be conjugated with ([2-(2-amino-ethoxy)-ethoxy]-acetyl)a-(gama-Glu)b-CO-(CH2)c-Z, wherein each a is independently an integer from 0 to 5, each b is independently an integer from 0 to 5, and each c is independently an integer from 10 to 24, wherein Z is independently selected from the group consisting of -CH3, carboxylic acids or carboxylic acid bioisosteres, phosphonates or sulfonates
  SITE 28: note = the epsilon-amino of the K side-chain may be conjugated with ([2-(2-amino-ethoxy)-ethoxy]-acetyl)a-(gama-Glu)b-CO-(CH2)c-Z, wherein each a is independently an integer from 0 to 5, each b is independently an integer from 0 to 5, and each c is independently an integer from 10 to 24, wherein Z is independently selected from the group consisting of -CH3, carboxylic acids or carboxylic acid bioisosteres, phosphonates or sulfonates
  SITE 40: note = the epsilon-amino of the K side-chain may be conjugated with ([2-(2-amino-ethoxy)-ethoxy]-acetyl)a-(gama-Glu)b-CO-(CH2)c-Z, wherein each a is independently an integer from 0 to 5, each b is independently an integer from 0 to 5, and each c is independently an integer from 10 to 24, wherein Z is independently selected from the group consisting of -CH3, carboxylic acids or carboxylic acid bioisosteres, phosphonates or sulfonates
YXEGTXTSDYXXXLDKXAQXEFVKWLLKXGPSSGAPPPSK